European Patent Application EP 4 431 101 A1, published September 18, 2024. Title: Therapeutic agent for chronic viral infections. Applicant: 公益財団法人東京都医学総合研究所. The sequence listing filed with the application follows.

SEQUENCE LISTING (10 sequences)

SEQ ID NO: 1 - DNA, 21 bp, synthetic construct
  source 1..21: mol_type = other DNA
cacatcaggattcctaggacc

SEQ ID NO: 2 - DNA, 20 bp, synthetic construct
  source 1..20: mol_type = other DNA
aggttggtgagtgattggag

SEQ ID NO: 3 - DNA, 26 bp, synthetic construct
  source 1..26: mol_type = other DNA
cagagtctagactcgtggtggacttc

SEQ ID NO: 4 - DNA, 25 bp, synthetic construct
  source 1..25: mol_type = other DNA
caaggcacagcttggaggcttgaac

SEQ ID NO: 5 - DNA, 25 bp, synthetic construct
  source 1..25: mol_type = other DNA
acggggcgcacctctctttacgcgg

SEQ ID NO: 6 - DNA, 26 bp, synthetic construct
  source 1..26: mol_type = other DNA
ccgtgtgcacttcgcttcacctctgc

SEQ ID NO: 7 - DNA, 21 bp, synthetic construct
  source 1..21: mol_type = other DNA
tggagatttttcagaggctgc

SEQ ID NO: 8 - DNA, 21 bp, synthetic construct
  source 1..21: mol_type = other DNA
aactccagcaagacctcttca

SEQ ID NO: 9 - DNA, 17 bp, synthetic construct
  source 1..17: mol_type = other DNA
gcacagagcctcgcctt

SEQ ID NO: 10 - DNA, 17 bp, synthetic construct
  source 1..17: mol_type = other DNA
ccttgcacatgccggag